European Patent Application EP 4 296 362 A1, published December 27, 2023. Title: Method for Producing Target Proteins. Applicant: National Institute of Advanced Industrial Science and Technology Asahi Kasei Pharma Corporation. The sequence listing filed with the application follows.

SEQUENCE LISTING (99 sequences)

SEQ ID NO: 1 - DNA, 864 bp, Burkholderia spp.
atgacctcgattagcaaacgtcatagccgccaacccgtcttccggcggattggcagcgggaccgaatttcggacaggcacagcggacgcgatagacgacgcgcccgaggcgtacgccccagacaggagggaggaactgcttgacgaaggggacgatgagtcccgtcgtccagtggactgcggccaggagaaggcgcttttcgaaggcgactcgtcgacgctaccgtatgacgtgcgccgggcgtacgcgctgcttcttcgcggtccatccattgacgaacgtcacagcaaactctggccagtcctgatcgatcatgaactgcgattgcgacagttgctacacgcggccttcctcgatctcgtcatcgatcgggagcaaaaaatcgcatttgcacgcccggtcgatgctccggagctcgacgtgccgcaacttctgcgggaggtccggcttactttcgttgattccgctctggtgcttttcctgaggatggagctgactctggctgaggccgaaggccgccgtgcaacggtttcccggtccgaaatggtcgatcatctcaaagcgtatgaagctagcgataatgttgaccgagcccgctttagcaggcaggtcgaggcggcgattgaaaaggccaagaaatacaacttccttcgcctgattcgtaatagcggagatcgcttcgaggtgtcgccagcgctcaagctggtgttctcacatgagcagataagcgaactgtcgcgaacctatcggcgtatcagggaacaggcggacggaagaccagcagaggtcgatggcgcggggagttttccgggcgtcgacgagccggacgaatttgacgaagacagtgtgatggacggggagtga

SEQ ID NO: 2 - protein, 287 aa, Burkholderia spp.
MTSISKRHSRQPAFRRMGGGTEFRTGIADVIDDAPEVSDLDGREELFDERDDEPHRPVDGGQERALFEGDSSTLPYDVRRAYALLLRGPSIDERHSRLWPVLIDHELRLRQLLHAAFLDLVIDREQKIAFARPVYAPELDVPQLLREVRLTFVDSALVLFLRMELTLAEAEGRRATISRSEMVDHLKAYEASDNVDRARFSRQVEAAIEKAKKYNFLRLIRNSGDRFEVSPALKLVFSHEQISELSLTYRRIREQADGRPAVDDGAGSMPSVDEPDEFDEDSVTDGE

SEQ ID NO: 3 - DNA, 3450 bp, Burkholderia spp.
gtggagacagcccagctattcgaggatccggaattgtcgccggcagcggcggacgagacggcgcataggggagaggatcatcgcccgacatggagcgattacgatctcgaagaagcggggcaacagcagttcaggctgcggcaaatgcaggtcatgaactgggggacgtttagcaagctccacgtattcgatatctcgccgcgcggacacttgctcgttgggccgtccggatcgggcaagtcgaccattctcgatgcgcattcggcgttgatggcgccgccgaattcagagttcaatgccgccgcccggggtaacgataaagtcacccgcgatcggacgatggtcacttatgtgcgcggggcttgggctacgcaggaatcggaggaagggatcatcgctgcgcagtacctgcggcctgacaccacccttagtgcagtcgccgaggtgtatgcaaacgcacaggggcagatgctgacgctggtcggcatgtggtggatcaagggtaagtcgacactcgcaaaggacgtgcgacactgtttcttcgtgatcgaacgggaattcagtctcaaggaactgtcgttcttcatgcaggccgactacaatctgcgctcgtttgcaaagcatcttccggaagtcaaacctttcgatacgcacgcgtccttccgtgaacgcttcaaggcgcgcctcggtatcgaccacgacctggcgttgcgactgcttcacaggacgcagtcgtcgaagaatctgggtgatatcaacgcgttcatgcgtgacaatatgctggacgagccccaaacgttcagcctcgccaaagcgctctgcgacgacttcaacacgctggcagcggcccaccaggacgtcgtggaggcccgtaagcagcgggacctgctgaacctcgcacgtttgcatcatgagctgtatcaggagcatcacacggaggtcgccagggtcgacgaactgctgaagcagctggaccatcaccgcgaatatctgcaatacacgttgcgtggcaggcgtgtggacgagttgaagattgtgctcaaagggctgcaccagagcgtcgatgcattggcccggaaggcgaacgacgagcagaccgaactccagcgattgatgacgcagcgtgccggcatgaacgacggcaatgtcgcaggactacagtcgcagttggccacgaaggaaacgcaactgaagcaggttcgccgtgcacgtgcacgggtgtcagtctggctccagacgctcgggtggcctgagccgcaagatgctggccattttggcgaatgtgtcggccgcgctggggtgctgcgggatcgtggtcagggcgaagaaggcgaggcaaaggccgaggaactgcgccagaagagatttgaggcagagcggcaactcaaggagctgctcgctgatgcggcatcgcttgaacagagaaaatcgaacttgccgcgagaactggtcaatgtccgtgaccagattgcacttgccctgaatctggatcccgcttcgcttccattcggcggtgaactgctcgacatatccgagaaattcaaacggtggcaaggtgttcttgagcgtttgctggctcctcttacccgctcgtttctcgtgccggaagaacactatccgggagttgtgaactggctcgagtcaaatcatacgggacagcatgtgctttacctgcgtatgcgcccgcatcagaagcgtttcgataatggtccgaaggctccgggcaggatgctggattcgtcggcggatgaatacggcgactggctgcgcgacgagatagccgtgcattacggcgactttgtgtgcgcagaaacgactgaagagtttcgcaattcgccacgcgccgtcagtctgcatggtcagatcaagcggggaggtgcacggcatgagaaaaatgaccgtacccgccttgatgaacgccggggctgggcgattggcttttccaacgagcagaaaaaacttgagcttctccatgaaattcacgctcagcagaaggtggaaagcgaagctagtcgggagttagccgaactcctggtgacgcagaacaaggaacgggagaagctgaacgcagcggcggaattgacgcaggtggtctgggaggacatcgacgacgtctcggtggccgatgaggtgcagcgtttgctgaaccagatagaagaggcgcaacggtcacacccggagatacaggaactcgatgggcaaatcaaggcgcagggggtaaaggcgtcccaggtgggtagcgcgcatgaaaccgaaaagaaaaaatacgctgatactgaacagcggatcaacgggttgacccgggatctggaaaatacacgtgacgatgtgcgtatgccgcctgtagatggggataagcttcagttattgtttggccacctggacggcctgacgctggagaacctggatcagcgacgcctgtctgcgcgcagcgaactgaaggacagaaggaacgacgccgataaggctcaagcaaatgaccggagcctgcttgaggaagtactccgtacgtttcagcgtgaacataagatggcggccgcggatatggggacgacgctggacgattggcccgactatgcccggctgttagccaaaatcgaggaggacgatctgccccgattcgaggagcggtttttcaggcttctcaacgagcagagcgatcgccatctggccagactgcggcagcgtctcgttaccgagaaggatgagatacgggggcgcatgaatattgtcaacgacgcactatcgcagactgagttcaacgctggcacctatctggttctggagaaccgccctcgaacgctgccggatgtgaccgcgttcctggccgaactcaagaactgccttgagcgcaatatcaaaccagatgcgacccgcgaagagcgcgaggagcagtttaaggcgctcaatacaatcgtccagcggttacacagtgacaagccggaggacgagcgttggaaagcactcgtcctcgacgtacggcaacacgtcgaatttgtggcgaaggaatttgatgctgatggtcgtgtgcgcgacatttttcagtccggcgccggtaagtctggcggacagcgacaaaagcttgccgcgacgtgcctcgcggcggcgctgcgctatcaactcgccgggacgcaaagaccgctgccgcagttttgcacggtattgatggatgaggcgttcgacaaagccgatagcgagttcacggcgatgacgctgaacatcttcaatacattcggattccagatgctgatggctacgccaatgaaggcagtaagaacgctcgaaccattcataggcggtgcacacgtctttagcaacaggttgcgcaacagttctggagcggtggcgatcgagtacgacatggcgcatcgacggctgctcggtctcagccaccagcgatccttagaaaaaggtaacgccgacggtgaaatgccgcagagcgaggactaa

SEQ ID NO: 4 - protein, 1149 aa, Burkholderia spp.
METAQLFEDPELSPVATDGAARREGEPRPTWSDRNLEEAGQQQFRLRQMQVMNWGTFSKLHVFDISPRGHLLVGPSGSGKSTILDAHSALMAPPNSEFNAAARGNDKVTRDRTMVTYVRGAWATQESEEGIIAAQYLRPDTTLSAVAEVYANAQGQMLTLVGMWWIKGKSTLAKDVRHCFFVIERAFSLKELSFFMQADYNLRSFAKHLPEVKPFDTHASFRERFKARLGIDHDLALRLLHRTQSSKNLGDINAFMRDNMLDEPQTFGLAKALCDDFNTLAAAHQDVVEAREQRDLLNLARSHHERYRAHHAEVARVDELLTQLDHHREYLQYTLRGRRVDELKIVLEGLRQSVDALARKANDDQTELQRLMTQRAGMNDGNVAGLQSQLVTKETQLKQVRRARARVSVWLQTLGWPEPQDAGHFGECVGRAGVLRDRGPGEEAEVKAEELRQKRFEAERQLKELLADAASLEQRKSNLPRELVNVRDQIALALNLDPASLPFGGELLDMPEKFRQWQGALERLLAPLTRSFLVPEEYYPGVVNWLESNHTGQHVLYLRMRPHQKRFDNGPKAPGRMLDSSADEYGGWLRNEIASHYGEFVCAETAEEFRNSPRAISLHGQIKRGGARHEKNDRTRLDERRHWVIGFSNEQKKLELLDEIHAQQKVEREASRALAELQATQNKEREKLNAAAELTQVVWEDIDDVSVADEVQHLLNQIEEAQRSHPEIQELDGQIQAQGVKASQAGSAHETEKKKFADTEQQINGLIRDRENTRDDVRMPPVDGDEIQLLFGHLDGLTLENLEQRRLSARSELKDRRNDADKAQANDRSLLEEVLRTFQREHKMAAADMGATLDDWSDYAQLLAKIEEDDLPRFEERFFRLLNEQSDRHLARLRQRLITEKDEIRGRMNIVNDALSQSEFNAGTYLVLENRPRTLPDVTAFLAELKSCLERNIRPEATREEREEQFKALNTIVQRLHSDKPEDERWKALVLDVRQHVEFVAKEFDADGRVRDIFQSGAGKSGGQRQKLAATCLAAALRYQLAGTQRPLPQFCTVLMDEAFDKADSEFTAMTLNIFNTFGFQMLMATPMKAVRTLEPFIGGAHVFSNKLRNSSGAVAIEYDMAHRRLVGLGHQRSEERGNAGGEIPQSED

SEQ ID NO: 5 - DNA, 1209 bp, Burkholderia spp.
atgccactggatgaacttggcggggcattgctgcccgacgatctcgcggttgcatgccggcgtcagctggagcgtcatcaggccggctggctggcgcagctatcggaggactcatggcccttatcggttgctttgcgtggtccgtcggacaggcaggcggtcaacgctccaggggccgtgcggacctggcttggtgcgtggaatgatttcgataggatttctagggaaaaggggcgaagggctgcggccgtgtggcgatcggtgaactggcggaccatgggcaacgtcaccataccggaaaaggtgttgttcgaagatgcgcaggctgtggcggattgtgcaggactgcgccggcattgggatacccttcatgcgcgctggcggaggataggcgagcggtatccggtcttggccggcgagcgcgattgcgcgaatgccgtcataagaaccgccgactggtctgacgatgatttccggcgactgatggaattgctggcctggtgcaggcagaacccggcgagcggactctacctgcgccaattgccactggtagacatagacacgaaatgggttgagggacggcgtggcgtcgtggaaccgctgcttcgaatccttatgggcaaggagggtgatattcgtgaggtcatggggctgaggcgttcacccgatacggtccggatgagactgctcgatgccgggcttcgcgagcaactgctgggcatggaggatattcagatccccgtaggccagtggaaccatgtgtttcggtatccaccaaagcgactactgattgtcgagaacctcgagtgcgggctggcgcttcccgatatcgaaggggtggcggtcgtgatggcgctcgggaacaatgtgactgccctacggggaatagaatgggcgcccgctgcggatgttctctactggggggacatcgatacctgggggttgcatattctgtcccgggctcgcggcatcttcccacatctgaggtcggttctgatgacggagggggtcgttgagtcgcatcgacatctcctgaccgacgagccgactcaggacaagcggcctgccgtgaatctcacgaaggacgaggcggaactattgtccgaccttcaaaccggacgatggggcgaacgccgtcgtctggaacaggagcgaatacactggccaaaggtaacagaggaagttcgccgccaatggacttattcttga

SEQ ID NO: 6 - protein, 402 aa, Burkholderia spp.
MPLGELGGALLPDDLAVACRRQLERHQADWLAQPSEGSWPLSVALRSPSDRQAANAPGAMRAWLGAWNDFDRISRDKGRRAAAVWRSVNWRTMGNVTIPERVLFEDAQAVADCAGLRRYWDTLHMRWQRMGERYPVLAGQRDCTNAVIRTADWSDDDFRRLMELLAWCRQNPASGLYLRQLPLIDIDTKWVEGRRGVVEPLVRILMGKDGDIREVMGLRRSPDTVRMRLLDPGLREQLLGMEDLQIPIGQWNHVFRYPPKRLLIVENLESGLALPDIEGVAVVMALGNNVTTLRGIEWALAADVLYWGDIDTWGLHILSRARGIFPHLRSVLMTEGVIESHRHLLTEEPTQDKRPAVNLTKDEAQLLSDLQAGRWGERRRLEQERIHWPNVIEEVCRQWTDS

SEQ ID NO: 7 - DNA, 90 bp, Burkholderia spp.
ttcgaactttactttttcgatttcgttcgttaaatttcgaattcgaacatttcgtgttcacccatttccatcagacgataaggacagcag

SEQ ID NO: 8 - DNA, 300 bp, Burkholderia spp.
gtcgcgcgcggtgccgccgcacgacgtctgcaggtcggcgaacgacggcgcccgccagttgccggcgagcggcggcgtgccggcgctgcaccccgccagaaggacggcgcacacgccggcccacatcccaatacgcatgattcacctcgcgaaacggtcgattccgccagtatcgtccgggatcgcgccgcgcgctactggccccgctttttcgaactttactttttcgatttcgttcgttaaatttcgaattcgaacatttcgtgttcacccatttccatcagacgataaggacagcag

SEQ ID NO: 9 - DNA, 110 bp, Burkholderia spp.
cagtgttttcgctctttcatggttttccctaggggacgccgggactaaactctgttccatcgctgcagacatggtgtgtgcggcggagcaaaaaaatcccggaggtaatc

SEQ ID NO: 10 - DNA, 300 bp, Burkholderia spp.
gctgccggcgaacctcgtgcaggcgcagcgcgacttcttcggcgcgcacacgttcgagcgtaccgacaagccgggcagcttccacgcgaactggtcgtaaccgcctcgcgggggcagcattgttgcgaaaatctattctatgaatagggtttctctatcccggatgccggcattgttggctccggggaaacagtgttttcgctctttcatggttttccctaggggacgccgggactaaactctgttccatcgctgcagacatggtgtgtgcggcggagcaaaaaaatcccggaggtaatc

SEQ ID NO: 11 - DNA, 966 bp, Burkholderia spp.
atggccgacgattacgcgacgacgcgttatccgatcgtcctcgtgcacgggctcacgggcaccgacaagtacgcgggcgtgctcgagtactggtacggcatccaggaagacctgcagcagcatggcgcgaccgtctacgtcgcgaacctgtcgggcttccagagcgacgacggcccgaacgggcgcggcgaacagttgctcgcgtacgtgaagacggtgcttgccgcgacgggcgcgaccaaggtcaatctcgtcggccacagccagggcgggctcacgtcgcgttacgtcgcggctgtcgcgccggatctcgtcgcgtcggtgacgacgatcggcacgccgcatcgcggctccgagttcgccgacttcgtgcagggcgtgctcgcatacgatccgaccgggctttcgtcatcggtgatcgcggcgttcgtcaatgtgttcggaatcctcacgagcagcagccacaacacgaaccaggacgcgctcgcgtcgctgaagacgctgacgaccgcccaggccgccacgtacaaccagaactatccgagcgcgggccttggcgcgccgggcagttgccagaccggcgcgccgacggaaaccgtcggcggcaacacgcatctgctgtattcgtgggccggcacggcgatccagccgacgctttccgtgttcggtgtcacgggcgcgacggacactagcacgattccgctcgtcgatccggcgaacgcgctcgacccgtcgacgcttgcgctgttcggcacgggcacggtgatgatcaaccgcggctcgggccagaacgacgggctcgtgtcgaaatgcagcgcgctgtacggccaggtgctgagcacgagctacaagtggaaccatatcgacgagatcaaccagttgctcggcgtgcgcggcgcgtttgcggaagatccggtcgcggtgatccgcacgcatgcgaaccgtctgaagctggcgggcgtgtaa

SEQ ID NO: 12 - DNA, 963 bp, Burkholderia spp.
atggcggacacctacgcggcgacgcgctatccggtgatcctcgtccacggcctcgcgggcaccgacaagttcgcgaacgtggtggactattggtacggaatccagagcgatctgcaatcgcatggcgcgaaggtgtacgtcgcgaatctctcgggattccagagcgacgacgggccgaacggccgcggcgagcagctgctcgcctacgtgaagcaggtgctcgcggccaccggcgcgaccaaggtgaacctgatcggccacagccagggcggcctgacctcgcgctacgtcgcggccgtcgcgccgcaactggtggcctcggtgacgacgatcggcacgccgcatcgcggctccgagttcgccgacttcgtgcaggacgtgctgaagaccgatccgaccgggctctcgtcgacggtgatcgccgccttcgtcaacgtgttcggcacgctcgtcagcagctcgcacaacaccgaccaggacgcgctcgcggcgctgcgcacgctcaccaccgcgcagaccgccacctacaaccggaacttcccgagcgcgggcctgggcgcgcccggttcgtgccagacgggcgccgcgaccgaaaccgtcggcggcagccagcacctgctctattcgtggggcggcaccgcgatccagcccacctccaccgtgctcggcgtgaccggcgcgaccgacaccagcaccggcacgctcgacgtcgcgaacgtgaccgacccgtccacgctcgcgctgctcgccaccggcgcggtgatgatcaatcgcgcctcggggcagaacgacgggctcgtctcgcgctgcagctcgctgttcgggcaggtgatcagcaccagctaccactggaaccatctcgacgagatcaaccagctgctcggcgtgcgcggcgccaacgcggaagatccggtcgcggtgatccgcacgcacgtgaaccggctcaagctgcagggcgtgtga

SEQ ID NO: 13 - DNA, 978 bp, Burkholderia spp.
atggcgagtgcgcccgtcgacaactacgcggcgacgcgttatccgatcattctcgtgcacgggctcacgggcaccgacaaatacgcaggtgtgctcgagtactggtatgggatccaggaggacctgcagcagcatggcgcgaccgtctatgtcgcgaacctgtcgggcttccagagcgacgacggcccgaacgggcgcggcgaacagttgctggcctacgtgaagacggtgctcgccgcgacgggggcgaccaaggtcaacctcgtcggtcacagccagggcgggctgacgtcgcgttatgtcgcggccgtcgcgcccgatctggtcgcgtcggtgacgacgatcggcacgccgcatcgcggctccgagttcgccgacttcgtgcagggcgtactcgcgtacgatccgaccgggctgtcgtcgacggtgatcgccgcgttcgtcaatgtgttcggaatcctcacgagcagcagcaacaacacgaaccaggacgcgctcgctgcgctgaagacgctgacgaccgcgcaggccgccacgtacaaccagaactacccgagcgcgggcctcggtgcgccgggcagttgccagaccggcgcgccgacggaaaccgtcggcggcaacacgcatctgttgtattcgtgggccggcaccgcgatccagccgacgatctccgtgttcggcgtcacgggtgcgacggatacgagcaccattccgctcgtcgatccggcgaatgcactcgacccgtcgacgctcgcgctgttcggcaccggcacggtgatgatcaaccgcggttcgggccagaacgacggagtcgtgtcgaagtgcagcgcgttgtacggccaggtgctgagcacgagctacaagtggaaccatctcgacgagatcaaccagttgctcggcgtgcgcggcgcgaatgcggaagatccggtcgcggtgatccgcacgcatgcgaaccggctgaagctcgcgggcgtgtga

SEQ ID NO: 14 - DNA, 1035 bp, Burkholderia spp.
atggcggcacgtgaagggcgcgcgccgctggcgcggcgcgctgcggtctacggtgtcgtggggctggcggcaatcgccggcgtcgcgatgtggagcggggcgggatggcatcgcggtgcgggtagcgccggcgaatcgcccgacgcggcggcggtgggcggcgtggctgcggcaccgccgcaggccgccgtgccggcgagcgcgggcctgccgtcgtcgctggccggttccagcgcgccgcggctgccgctcgatgcgggcggccatctcgcgaaggtacgcgcggtgcgcgatttcttcgactactgcctgaccgcgcagagcgacctcagcgcggccgcgctcgacgcactcgtcgtgcgcgagattgccgcgcagctcgacggcacggccgcgcacgccgaggcgctcgacgtgtggcatcgttatcgcgcgtatctcgacgcgctcgcgaaactgcgcgatgccggcgcggtcgacaagtccgatttgggcgcgctgcaactcgcgctcgaccagcgcgcatcgatcgcgtatcgcacgcttggcgactggagccagccgttcttcggcgcggaacagtggcggcagcgctacgatctcgcgcggctgaagatcgcgcaggatcgcacgctgaccgatgcgcagaaggccgagcggctcgcggcgctggagcagcagctgccggccgatgaacgcgccgcgcagcagcgggtcgaccggcagcgggccgcgatcgaccagatcgcgcagttgcagaagaacggggcgacgcccgatgcgatgcgcgcgcaactgacgcagacgctcgggcccgaggccgccgcgcgcgtcgcgcagatgcagcacgacgacgcatcgtggcagagccgctacgcggactatgcggcgcagcgtgcgcagatcgaatcggccggcctgtcgccgcaggaccgcgacgcgcagatcgccgcgttgcggcagcgcgtgttcacgaaacccggcgaagcggtgcgcgcggcgtcgctcgatcgcggggcgggcagcgcgcagtaa

SEQ ID NO: 15 - DNA, 1062 bp, Burkholderia spp.
atggcgcaggccgatcgtccggcgcgcggcgggctggccgcgcgcccgatgcgcggcgcgtcgttcgcgctggccgggctcgtcgcgtgtgccgcctgtgccgcggtcgtgctgtggcttcggcccgccgccccgtcgcccgcgccggccggcgccgtcgcgggcgggccggcggccggcgtgcccgccgcggcaagcggcgcggcggaggccgccatgccgttgccggcggcgctgccgggcgcgctggctggctcgcatgcgccgcgcctgccgctggccgccggcggccggctcgcgaggacgcgcgcggtgcgcgagttcttcgactattgcctgaccgcgcagggcgaactgacgcccgccgcgctcgatgcgctggtgcggcgcgagatcgccgcgcagcttgacggcagccccgcgcaagcggaggcgctcggcgtctggcgccgctatcgcgcctacttcgacgcgctcgcgcaattgcccggcgacggcgcggtgctcggcgacaagctcgatccggccgccatgcagctcgcgctcgatcagcgcgcggcgctggccgaccgcacgctcggcgagtgggccgagccgttcttcggcgacgagcagcgccggcagcgccatgacctcgaacggatccggatcgccaacgacaccacgctgagccctgagcagaaggccgcgcggcttgccgcgctcgacgcgcagctgacgccggacgagcgcgcgcagcaggcggcgctgcatgcgcagcaggacgcggtgacgaagatcgccgacttgcagaaggccggcgcgacgcccgaccagatgcgcgcgcagatcgcgcagacgctcgggcccgaggcggccgcgcgcgccgcgcagatgcagcaggacgacgaggcgtggcagacgcgctatcaagcctatgcggccgagcgcgaccggatcgcggcgcaggggctcgcgccgcaggatcgcgatgcgcggatcgcgcagctcaggcagcagactttcacggcgccgggggaggcgatccgcgcggcgtcgctcgatcgcggcgcgggcggttag

SEQ ID NO: 16 - DNA, 1035 bp, Burkholderia spp.
atgacggcacgtgaagggcgcgcgccgctggcgcggcgcgctgtggtctacggtgtcgtggggctggcggcgatcgccggcgtcgcgatgtggagcggtgcgggatggcatcgcgggacgggcacggccgccgagttgccggacgcggctgcggcaggcggggcggctgccgcgccgccgcagggcgccatgccggcgagcacgggcctgccgtcgtcgctggccggctccagcgcgccgcgactgccgctcgatgccggcggccatcttgcgaagtcgcgtgtggtgcgcgatttcttcgactactgcctgaccgcgcagagcgacctgagcgcggccgcgctcgatgcgttcgtcgtacgcgagatcgccgcgcagctcgacggcacggttgcgcaggccgaggcgctcgacgtctggcaccggtaccgtgcgtatctcgacgcgctcgcgaagttgcgcgatgccggcgcggtcgacaagtccgacctgggcgcgctgcagctcgcgctcgaccagcgcgcgtcgatcgcataccgcacgctcggcgactggagccagccgtttttcggcgcggagcagtggcggcagcgctacgatctcgcgcgattgaagatcgcacaggatcgcacgctgacggatgcgcagaaggccgagcggctcgcggcgctcgagcagcagatgccggccgacgagcgcgccgcgcagcagcgggtcgaccagcagcgggccgcgatcgaccagatcgcgcaattgcagaagggcggcgcgacgcccgatgcgatgcgcgcgcaactgacgcagacgctcggcccggaagccgccgcgcgcgtcgcgcagatgcagcaggacaacgcatcgtggcagagccgctacgcggactatgcggcgcagcgtgcgcagatcgagtcggccggcctgtcgccgcaggatcgcgatgcacagatcgccgcgttacgacagcgcgtgttcacgaaacccggtgaggccgtgcgggcggcatcgctcgatcgcggcgcgggcagcgcgcagtga

SEQ ID NO: 17 - DNA, 21 bp, Artificial Sequence
  Primer
gcaattccacgtctaccgatg

SEQ ID NO: 18 - DNA, 29 bp, Artificial Sequence
  Priner
tgctttacctccgctaagtggtgatgaac

SEQ ID NO: 19 - DNA, 257 bp, Artificial Sequence
  Amplified product
gcaattccacgtctaccgatggctcgggtggttctgacggctgcgcggaaacgggagcggaatggcagccccacccaggatggcaggcgcgtgacgaagtgcacgaagtgttgcgcgacttcaacgcggccttgcgttgcgccaagatccggtgcacattgatccgtcacttttgttacactcgacacgcactcgtttgcagtcgccagacaaaacggcaacattcgggttcatcaccacttagcggaggtaaagca

SEQ ID NO: 20 - DNA, 32 bp, Artificial Sequence
  Primer
atgaacatcaaaaagtttgcaaaacaagcaac

SEQ ID NO: 21 - DNA, 29 bp, Artificial Sequence
  Primer
atgggttaaaaaggatcgatcctctagcg

SEQ ID NO: 22 - DNA, 35 bp, Artificial Sequence
  Amplified product
acatgattacgaattggcgcatgaatattgtcaac

SEQ ID NO: 23 - DNA, 35 bp, Artificial Sequence
  Primer
ccagccggcctgatgacgctccagctgacgccggc

SEQ ID NO: 24 - DNA, 35 bp, Artificial Sequence
  Primer
catcaggccggctggcgatggggcgaacgccgtcg

SEQ ID NO: 25 - DNA, 35 bp, Artificial Sequence
  Primer
ggccagtgccaagcttccgccgaagtcgtggatac

SEQ ID NO: 26 - DNA, 35 bp, Artificial Sequence
  Primer
acatgattacgaattccggacaagatggcgttgtg

SEQ ID NO: 27 - DNA, 27 bp, Artificial Sequence
  Primer
tgtcgggcgatgatcctctcccctatg

SEQ ID NO: 28 - DNA, 35 bp, Artificial Sequence
  Primer
gatcatcgcccgacaatggcgcatcgacggctgct

SEQ ID NO: 29 - DNA, 35 bp, Artificial Sequence
  Primer
ggccagtgccaagctcgtagggcagtcacattgtt

SEQ ID NO: 30 - DNA, 35 bp, Artificial Sequence
  Primer
acatgattacgaattgatgactgaggcgattgcag

SEQ ID NO: 31 - DNA, 31 bp, Artificial Sequence
  Primer
cgcgtccgctgtgcctgtccgaaattcggtc

SEQ ID NO: 32 - DNA, 35 bp, Artificial Sequence
  Primer
ggcacagcggacgcgagaccagcagaggtcgatgg

SEQ ID NO: 33 - DNA, 35 bp, Artificial Sequence
  Primer
ggccagtgccaagctccgtgtgatgctcctgatac

SEQ ID NO: 34 - DNA, 20 bp, Artificial Sequence
  Primer
ggcgcatgaatattgtcaac

SEQ ID NO: 35 - DNA, 20 bp, Artificial Sequence
  Primer
tccgccgaagtcgtggatac

SEQ ID NO: 36 - DNA, 20 bp, Artificial Sequence
  Primer
ccggacaagatggcgttgtg

SEQ ID NO: 37 - DNA, 20 bp, Artificial Sequence
  Primer
cgtagggcagtcacattgtt

SEQ ID NO: 38 - DNA, 20 bp, Artificial Sequence
  Primer
gatgactgaggcgattgcag

SEQ ID NO: 39 - DNA, 20 bp, Artificial Sequence
  Primer
ccgtgtgatgctcctgatac

SEQ ID NO: 40 - DNA, 26 bp, Artificial Sequence
  Primer
gctgaaagcttacctgagcttaaaag

SEQ ID NO: 41 - DNA, 26 bp, Artificial Sequence
  Primer
cagcgtgttcagcattattccatttg

SEQ ID NO: 42 - DNA, 32 bp, Artificial Sequence
  Primer
cgttaaatattgcagcatgcgcgcgcacgaac

SEQ ID NO: 43 - DNA, 29 bp, Artificial Sequence
  Primer
gcagatctggccaacgtttgcgccctgac

SEQ ID NO: 44 - DNA, 50 bp, Artificial Sequence
  Primer
caaacgttggccagatctgctagctacgtagagctcggtaccactagtgg

SEQ ID NO: 45 - DNA, 47 bp, Artificial Sequence
  Primer
aaaccgcggccatatgggtctagaggatccactagtggtaccgagct

SEQ ID NO: 46 - DNA, 32 bp, Artificial Sequence
  Primer
ccatatggccgcggttttcgactgcttcaaag

SEQ ID NO: 47 - DNA, 31 bp, Artificial Sequence
  Primer
cataagcggccgggcgacgaggccagagagc

SEQ ID NO: 48 - DNA, 87 bp, Artificial Sequence
  Terminator
gccgcggttttcgactgcttcaaagccccgctccggcggggctttttcattgatgcccgtccgggcgctctctggcctcgtcgcccg

SEQ ID NO: 49 - DNA, 97 bp, Artificial Sequence
  Terminator
ttgcagcatgcgcgcgcacgaacgcggccccgcccgaacgggcggggcgcgtcaagcgattagagaaccgtgtctagtcagggcgcaaacgttggcc

SEQ ID NO: 50 - DNA, 56 bp, Artificial Sequence
  MCS fragment
agatctgctagctacgtagagctcggtaccactagtggatcctctagacccatatg

SEQ ID NO: 51 - DNA, 37 bp, Artificial Sequence
  Primer
tcgtcgcccggccgcttatgtctattgctggtttacc

SEQ ID NO: 52 - DNA, 36 bp, Artificial Sequence
  Primer
gcatgctgcaatatttaacgaccctgccctgaaccg

SEQ ID NO: 53 - DNA, 24 bp, Artificial Sequence
  Primer
gccagatcgatgcgttccagggtg

SEQ ID NO: 54 - DNA, 30 bp, Artificial Sequence
  Primer
cataagcggcttactgcgcgctgcccgccc

SEQ ID NO: 55 - DNA, 40 bp, Artificial Sequence
  Primer
acgttggccagatctgcaattccacgtctaccgatggctc

SEQ ID NO: 56 - DNA, 44 bp, Artificial Sequence
  Primer
acgcatcgatctggccattgctttacctccgctaagtggtgatg

SEQ ID NO: 57 - DNA, 32 bp, Artificial Sequence
  Primer
gcagtaagccgcggttttcgactgcttcaaag

SEQ ID NO: 58 - DNA, 25 bp, Artificial Sequence
  Primer
agatctggccaacgtttgcgccctg

SEQ ID NO: 59 - DNA, 35 bp, Artificial Sequence
  Primer
accactgcgatccccactggatgacggcgatgacc

SEQ ID NO: 60 - DNA, 35 bp, Artificial Sequence
  Primer
gaatgctgttttcccgtcgatgtcgaggatggcgg

SEQ ID NO: 61 - DNA, 20 bp, Artificial Sequence
  Primer
actggatgacggcgatgacc

SEQ ID NO: 62 - DNA, 23 bp, Artificial Sequence
  Primer
gtcgatgtcgaggatggcggaag

SEQ ID NO: 63 - DNA, 20 bp, Artificial Sequence
  Primer
ctgtggccgatctagggctg

SEQ ID NO: 64 - DNA, 20 bp, Artificial Sequence
  Primer
acgcgctttgagattcccag

SEQ ID NO: 65 - DNA, 5376 bp, Artificial Sequence
  pSa plasmid
gctgtagccgcctcgccgccctataccttgtctgcctccccgcgttgcgtcgcggtgcatggagccgggccacctcgacctgaatggaagccggcggcacctcgctaacggattcaccgtttttatcaggctctgggaggcagaataaatgatcatatcgtcaattattacctccacggggagagcctgagcaaactggcctcaggcatttgagaagcacacggtcacactgcttccggtagtcaataaaccggtaaaccagcaatagacataagcggctatttaacgaccctgccctgaaccgacgaccgggtcgaatttgctttcgaatttctgccattcatccgcttattatacttattcaggcgtagcaccaggcgtttaagggcaccaataactgccttaaaaaaattacgccccgccctgccactcatcgcagtactgttgtaattcattaagcattctgccgacatggaagccatcacagacggcatgatgaacctgaatcgccagcggcatcagcaccttgtcgccttgcgtataatatttgcccatggtgaaaacgggggcgaagaagttgtccatattggccacgtttaaatcaaaactggtgaaactcacccagggattggctgagacgaaaaacatattctcaataaaccctttagggaaataggccaggttttcaccgtaacacgccacatcttgcgaatatatgtgtagaaactgccggaaatcgtcgtggtattcactccagagcgatgaaaacgtttcagtttgctcatggaaaacggtgtaacaagggtgaacactatcccatatcaccagctcaccgtctttcattgccatacggaattccggatgagcattcatcaggcgggcaagaatgtgaataaaggccggataaaacttgtgcttatttttctttacggtctttaaaaaggccgtaatatccagctgaacggtctggttataggtacattgagcaactgactgaaatgcctcaaaatgttctttacgatgccattgggatatatcaacggtggtatatccagtgatttttttctccattttagcttccttagctcctgaaaatctcgataactcaaaaaatacgcccggtagtgatcttatttcattatggtgaaagttggaacctcttacgtgccgatcaacgtctcattttcgccaaaagttggcccagggcttcccggtatcaacagggacaccaggatttatttattctgacaggctgcgcctgcccacgagcttgaccacagggattgcccaccggctacccagccttcgaccacatacccaccggctccaactgcgcggcctgcggccttgccccatcaatttttttaattttctctggggaaaagcctccggcctgcggcctgcgcgcttcgcttgccggttggacaccaagtggaaggcgggtcaaggctcgcgcagcgaccgcgcagcggcttggccttgacgcgcctggaacgacccaagcctatgcgagtgggggcagtcgaaggcgaagcccgcccgcctgccccccgagacctgcaggggggggggggcgctgaggtctgcctcgtgaagaaggtgttgctgactcataccaggcctgaatcgccccatcatccagccagaaagtgagggagccacggttgatgagagctttgttgtaggtggaccagttggtgattttgaacttttgctttgccacggaacggtctgcgttgtcgggaagatgcgtgatctgatccttcaactcagcaaaagttcgatttattcaacaaagccgccgtcccgtcaagtcagcgtaatgctctgccagtgttacaaccaattaaccaattctgattagaaaaactcatcgagcatcaaatgaaactgcaatttattcatatcaggattatcaataccatatttttgaaaaagccgtttctgtaatgaaggagaaaactcaccgaggcagttccataggatggcaagatcctggtatcggtctgcgattccgactcgtccaacatcaatacaacctattaatttcccctcgtcaaaaataaggttatcaagtgagaaatcaccatgagtgacgactgaatccggtgagaatggcaaaagcttatgcatttctttccagacttgttcaacaggccagccattacgctcgtcatcaaaatcactcgcatcaaccaaaccgttattcattcgtgattgcgcctgagcgagacgaaatacgcgatcgctgttaaaaggacaattacaaacaggaatcgaatgcaaccggcgcaggaacactgccagcgcatcaacaatattttcacctgaatcaggatattcttctaatacctggaatgctgttttcccggggatcgcagtggtgagtaaccatgcatcatcaggagtacggataaaatgcttgatggtcggaagaggcataaattccgtcagccagtttagtctgaccatctcatctgtaacatcattggcaacgctacctttgccatgtttcagaaacaactctggcgcatcgggcttcccatacaatcgatagattgtcgcacctgattgcccgacattatcgcgagcccatttatacccatataaatcagcatccatgttggaatttaatcgcggcctcgagcaagacgtttcccgttgaatatggctcataacaccccttgtattactgtttatgtaagcagacagttttattgttcatgatgatatatttttatcttgtgcaatgtaacatcagagattttgagacacaacgtggctttcccccccccccctgcaggtcccgagcctcacggcggcgagtgcgggggttccaagggggcagcgccaccttgggcaaggccgaaggccgcgcagtcgatcaacaagccccggaggggccactttttgccggagggggagccgcgccgaaggcgtgggggaaccccgcaggggtgcccttagtcaaaagcctccgaccggaggcttttgactaaaacttcccttggggttatcattggggctcactcaaaggcggtaatcagataaaaaaaatccttagctttcgctaaggatgatttctgctagagctgtcagaccagagctccaaaccaacgttttatctataccgctacagggtatttaattcctatttaatctgcgctagaatgaggcatgtttaaccgaatctgacgttttccctgcaaatgccaaaatactatgcctatctccgggtttcgcgtgacggccaagacccggaaaaccaaaaatacggtttgctcgaatacgcgaacgccaaaggcttcgcgccgctacagatcgaggaagaaattgccagcagagcaaaggactggcgcaagcgcaagctcggagcaatcatcgaaaaggccgagcgtggcgacgtgctactgacgccggagattacgcgcattgccggttccgccctcgccgccttggaaattctcaaagcggcgagcgagcgcggcctaatcgtccatgtgaccaaacagaagatcatcatggacggcagcctacaaagcgacatcatggcaaccgtgcttggcttggctgcacagatcgagcggcatttcattcaggcacgtaccaccgaggcgctacaagtcgccagagagcgcggcaagacgctcgggcgacccaagggcagcaaatcgagcgccttgaagctggacagccgtattgatgaagtacaggcatacgtgaaccttggcttgccgcaaagtcgcgcagccgagttgttaggcgtcagccctcacaccttgcgcctgttcatcaaacgccggaacatcaaacccacaaacactagaccaaccatcaccatgccggggagggaacaacatgcctaagaacaacaaagcccccggccatcgtatcaacgagatcatcaagacgagcctcgcgctcgaaatggaggatgcccgcgaagctggcttagtcggctacatggcccgttgccttgtgcaagcgaccatgccccacaccgaccccaagaccagctactttgagcgcaccaatggcatcgtcaccttgtcgatcatgggcaagccgagcatcggcctgccctacggttctatgccgcgcaccttgcttgcttggatatgcaccgaggccgtgcgaacgaaagaccccgtgttgaaccttggccggtcgcaatcggaatttctacaaaggctcggaatgcacaccgatggccgttacacggccacccttcgcaatcaggcgcaacgcctgttttcatccatgatttcgcttgccggcgagcaaggcaatgacttcggcattgagaacgtcgtcattgccaagcgcgcttttctattctggaatcccaagcggccagaagatcgggcgctatgggatagcaccctcaccctcacaggcgatttcttcgaggaagtcacccgctcaccggttcctatccgaatcgactacctgcatgccttgcggcagtctccgcttgcgatggacatttacacgtggctgacctatcgcgtgttcctgttgcgggccaagggccgccccttcgtgcaaatcccttgggtcgccctgcaagcgcaattcggctcatcctatggcagccgcgcacgcaactcgcccgaactggacgataaggcccgagagcgggcagagcgggcagcactcgccagcttcaaatacaacttcaaaaagcgcctacgcgaagtgttgattgtctatcccgaggcaagcgactgcatcgaagatgacggcgaatgcctgcgcatcaaatccacacgcctgcatgtcacccgcgcacccggcaagggcgctcgcatcggcccccctccgacttgaccaggccaacgctacgcttggcttggtcaagccttcccatccaacagcccgccgtcgagcgggcttttttatccccggaagcctgtggatagagggtagttatccacgtgaaaccgctaatgccccgcaaagccttgattcacggggctttccggcccgctccaaaaactatccacgtgaaatcgctaatcagggtacgtgaaatcgctaatcggagtacgtgaaatcgctaataaggtcacgtgaaatcgctaatcaaaaaggcacgtgagaacgctaatagccctttcagatcaacagcttgcaaacacccctcgctccggcaagtagttacagcaagtagtatgttcaattagcttttcaattatgaatatatatatcaattattggtcgcccttggcttgtggacaatgcgctacgcgcaccggctccgcccgtggacaaccgcaagcggttgcccaccgtcgagcgccagcgcctttgcccacaacccggcggccgcaacagatcgttttataaatttttttttttgaaaaagaaaaagcc

SEQ ID NO: 66 - DNA, 6475 bp, Artificial Sequence
  pRK2-182 plasmid
aaagccacgttgtgtctcaaaatctctgatgttacattgcacaagataaaaatatatcatcatgaacaataaaactgtctgcttacataaacagtaatacaaggggtgttatgagccatattcaacgggaaacgtcttgctcgaggccgcgattaaattccaacatggatgctgatttatatgggtataaatgggctcgcgataatgtcgggcaatcaggtgcgacaatctatcgattgtatgggaagcccgatgcgccagagttgtttctgaaacatggcaaaggtagcgttgccaatgatgttacagatgagatggtcagactaaactggctgacggaatttatgcctcttccgaccatcaagcattttatccgtactcctgatgatgcatggttactcaccactgcgatccccgggaaaacagcattccaggtattagaagaatatcctgattcaggtgaaaatattgttgatgcgctggcagtgttcctgcgccggttgcattcgattcctgtttgtaattgtccttttaacagcgatcgcgtatttcgtctcgctcaggcgcaatcacgaatgaataacggtttggttgatgcgagtgattttgatgacgagcgtaatggctggcctgttgaacaagtctggaaagaaatgcataagcttttgccattctcaccggattcagtcgtcactcatggtgatttctcacttgataaccttatttttgacgaggggaaattaataggttgtattgatgttggacgagtcggaatcgcagaccgataccaggatcttgccatcctatggaactgcctcggtgagttttctccttcattacagaaacggctttttcaaaaatatggtattgataatcctgatatgaataaattgcagtttcatttgatgctcgatgagtttttctaatcagaattggttaattggttgtaacactggcagagcattacgctgacttgacgggacggcggctttgttgaataaatcgaacttttgctgagttgaaggatcagatcacgcatcttcccgacaacgcagaccgttccgtgctgagcgtcagaccccgtagaaaagatcaaaggatcttcttgagatcctttttttctgcgggggatcaggaccgctgccggagcgcaacccactcactacagcagagccatgtagggccgccggcgttgtggataccacgcggaaaacttggccctcactgacagatgaggggcggacgttgacacttgaggggccgactcacccggcgcggcgttgacagatgaggggcaggctcgatttcggccggcgacgtggagctggccagcctcgcaaatcggcgaaaacgcctgattttacgcgagtttcccacagatgatgtggacaagcctggggataagtgccctgcggtattgacacttgaggggcgcgactactgacagatgaggggcgcgatccttgacacttgaggggcagagtgatgacagatgaggggcgcacctattgacatttgaggggctgtccacaggcagaaaatccagcatttgcaagggtttccgcccgtttttcggccaccgctaacctgtcttttaacctgcttttaaaccaatatttataaaccttgtttttaaccagggctgcgccctggcgcgtgaccgcgcacgccgaaggggggtgcccccccttctcgaaccctcccggcccgctaacgcggcaccccatccccccaggggctgcgcccctcggccgcgaacgacctcaccccaaaaatggcagccacgtagaaagccagtccgcagaaacggtgctgaccccggatgaatgtcagctactgggctatctggacaagggaaaacgcaagcgcaaagagaaagcaggtagcttgcagtgggcttacatggcgatagctagactgggcggttttatggacagcaagcgaaccggaattgccagctggggcgccctctggtaaggttgggaagccctgcaaagtaaactggatggctttcttgccgccaaggatctgatggcgcaggggatcaagatcgacggatcgatccggggaattaattccggggcaatcccgcaaggagggtgaatgaatcggacgtttgaccggaaggcatacaggcaagaactgatcgacgcggggttttccgccgaggatgccgaaaccatcgcaagccgcaccgtcatgcgtgcgccccgcgaaaccttccagtccgtcggctcgatggtccagcaagctacggccaagatcgagcgcgacagcgtgcaactggctccccctgccctgcccgcgccatcggccgccgtggagcgttcgcgtcgtctcgaacaggaggcggcaggtttggcgaagtcgatgaccatcgacacgcgaggaactatgacgaccaagaagcgaaaaaccgccggcgaggacctggcaaaacaggtcagcgaggccaagcaggccgcgttgctgaaacacacgaagcagcagatcaaggaaatgcagctttccttgttcgatattgcgccgtggccggacacgatgcgagcgatgccaaacgacacggcccgctctgccctgttcaccacgcgcaacaagaaaatcccgcgcgaggcgctgcaaaacaaggtcattttccacgtcaacaaggacgtgaagatcacctacaccggcgtcgagctgcgggccgacgatgacgaactggtgtggcagcaggtgttggagtacgcgaagcgcacccctatcggcgagccgatcaccttcacgttctacgagctttgccaggacctgggctggtcgatcaatggccggtattacacgaaggccgaggaatgcctgtcgcgcctacaggcgacggcgatgggcttcacgtccgaccgcgttgggcacctggaatcggtgtcgctgctgcaccgcttccgcgtcctggaccgtggcaagaaaacgtcccgttgccaggtcctgatcgacgaggaaatcgtcgtgctgtttgctggcgaccactacacgaaattcatatgggagaagtaccgcaagctgtcgccgacggcccgacggatgttcgactatttcagctcgcaccgggagccgtacccgctcaagctggaaaccttccgcctcatgtgcggatcggattccacccgcgtgaagaagtggcgcgagcaggtcggcgaagcctgcgaagagttgcgaggcagcggcctggtggaacacgcctgggtcaatgatgacctggtgcattgcaaacgctagggccttgtggggtcagttccggctgggggttcagcagccacctgcatcgcaagctagcttgctagagggtcagctttatgcttgtaaaccgttttgtgaaaaaatttttaaaataaaaaaggggacctctagggtccccaattaattagtaatataatctattaaaggtcattcaaaaggtcatccaccggatcaattcccctgctcgcgcaggctgggtgccaagctctcgggtaacatcaaggcccgatccttggtagtcggcaaataatgtctaacaattcgttcaagccgacgccgcttcgcggcgcggcttaactcaagcgttagatgcactaagcacataattgctcacagccaaactatcaggtcaagtctgcttttattatttttaagcgtgcataataagccctacacaaattgggagatatatcatgaaaggctggctttttcttgttatcgcaatagttggcgaagtaatcgcaacatccgcattaaaatctagcgagggctttactaagctgatccggtggatgaccttttgaatgacctttaatagattatattactaattaattggggaccctagaggtccccttttttattttaaaaattttttcacaaaacggtttacaagcataaagctgactctagctagaggatcttcgaatgcatcgcgcgcaccgtacgtctcgaggaattcgcaattccacgtctaccgatggctcgggtggttctgacggctgcgcggaaacgggagcggaatggcagccccacccaggatggcaggcgcgtgacgaagtgcacgaagtgttgcgcgacttcaacgcggccttgcgttgcgccaagatccggtgcacattgatccgtcacttttgttacactcgacacgcactcgtttgcagtcgccagacaaaacggcaacattcgggttcatcaccacttagcggaggtaaagcaatggccagatcgatgcgttccagggtggtggcaggggcagtggcatgcgcgatgagcgtcgcgccgttcgcggggacgaccgcggtgatgacgctcgcgacgacgcacgcggcgatggcggcgaccgcgcccgccgacgattacgcgacgacgcgttatccgatcgtcctcgtgcacgggctcacgggcaccgacaagtacgcgggcgtgctcgagtactggtacggcatccaggaagacctgcagcagcatggcgcgaccgtctacgtcgcgaacctgtcgggcttccagagcgacgacggcccgaacgggcgcggcgaacagttgctcgcgtacgtgaagacggtgcttgccgcgacgggcgcgaccaaggtcaatctcgtcggccacagccagggcgggctcacgtcgcgttacgtcgcggctgtcgcgccggatctcgtcgcgtcggtgacgacgatcggcacgccgcatcgcggctccgagttcgccgacttcgtgcagggcgtgctcgcatacgatccgaccgggctttcgtcatcggtgatcgcggcgttcgtcaatgtgttcggaatcctcacgagcagcagccacaacacgaaccaggacgcgctcgcgtcgctgaagacgctgacgaccgcccaggccgccacgtacaaccagaactatccgagcgcgggccttggcgcgccgggcagttgccagaccggcgcgccgacggaaaccgtcggcggcaacacgcatctgctgtattcgtgggccggcacggcgatccagccgacgctttccgtgttcggtgtcacgggcgcgacggacactagcacgattccgctcgtcgatccggcgaacgcgctcgacccgtcgacgcttgcgctgttcggcacgggcacggtgatgatcaaccgcggctcgggccagaacgacgggctcgtgtcgaaatgcagcgcgctgtacggccaggtgctgagcacgagctacaagtggaaccatatcgacgagatcaaccagttgctcggcgtgcgcggcgcgtttgcggaagatccggtcgcggtgatccgcacgcatgcgaaccgtctgaagctggcgggcgtgtaatcgatggcggcacgtgaagggcgcgcgccgctggcgcggcgcgctgcggtctacggtgtcgtggggctggcggcaatcgccggcgtcgcgatgtggagcggggcgggatggcatcgcggtgcgggtagcgccggcgaatcgcccgacgcggcggcggtgggcggcgtggctgcggcaccgccgcaggccgccgtgccggcgagcgcgggcctgccgtcgtcgctggccggttccagcgcgccgcggctgccgctcgatgcgggcggccatctcgcgaaggtacgcgcggtgcgcgatttcttcgactactgcctgaccgcgcagagcgacctcagcgcggccgcgctcgacgcactcgtcgtgcgcgagattgccgcgcagctcgacggcacggccgcgcacgccgaggcgctcgacgtgtggcatcgttatcgcgcgtatctcgacgcgctcgcgaaactgcgcgatgccggcgcggtcgacaagtccgatttgggcgcgctgcaactcgcgctcgaccagcgcgcatcgatcgcgtatcgcacgcttggcgactggagccagccgttcttcggcgcggaacagtggcggcagcgctacgatctcgcgcggctgaagatcgcgcaggatcgcacgctgaccgatgcgcagaaggccgagcggctcgcggcgctggagcagcagctgccggccgatgaacgcgccgcgcagcagcgggtcgaccggcagcgggccgcgatcgaccagatcgcgcagttgcagaagaacggggcgacgcccgatgcgatgcgcgcgcaactgacgcagacgctcgggcccgaggccgccgcgcgcgtcgcgcagatgcagcacgacgacgcatcgtggcagagccgctacgcggactatgcggcgcagcgtgcgcagatcgaatcggccggcctgtcgccgcaggaccgcgacgcgcagatcgccgcgttgcggcagcgcgtgttcacgaaacccggcgaagcggtgcgcgcggcgtcgctcgatcgcggggcgggcagcgcgcagtaagccgcggttttcgactgcttcaaagccccgctccggcggggctttttcattgatgcccgtccgggcgctctctggcctcgtcgcccgtctagatacctaggtgagctctggtaccgcggccgcaattcac

SEQ ID NO: 67 - DNA, 2138 bp, Burkholderia plantarii
atggtcagatcgatgcgttccagggtggcggcgagggcggtggcatgggcgttggcggtgatgccgctggccggcgcggccgggttgacgatggccgcgtcgcccgcggccgtcgcggcggacacctacgcggcgacgcgctatccggtgatcctcgtccacggcctcgcgggcaccgacaagttcgcgaacgtggtggactattggtacggaatccagagtgatctgcaatcgcatggcgcgaaggtgtacgtcgcgaatctctcgggattccagagcgacgacgggccgaacggccgcggcgagcagctgctcgcctacgtgaagcaggtgctcgcggccaccggcgcgaccaaggtgaacctgatcggccacagccagggcggcctgacctcgcgctacgtcgcggccgtggcgccgcaactggtggcgtcggtgacgacgatcggcacgccgcatcgcggctccgagttcgccgacttcgtgcaggacgtgctgaagaccgatccgaccgggctctcgtcgacggtgatcgccgccttcgtcaacgtgttcggcacgctcgtcagcagctcgcacaacaccgaccaggatgcgctcgcggcgctgcgcacgctcaccaccgcgcagaccgccacctacaaccggaacttcccgagcgcgggcctgggcgcgcccggttcgtgccagacgggcgccgcgaccgaaaccgtcggcggcagccagcacctgctctattcgtggggcggcaccgcgatccagcccacctccaccgtgctcggcgtgaccggcgcgaccgacaccagcaccggcacgctcgacgtcgcgaacgtgaccgacccgtccacgctcgcgctgctcgccaccggcgcggtgatgatcaatcgcgcctcggggcagaacgacgggctcgtctcgcgctgcagctcgctgttcgggcaggtgatcagcaccagctaccactggaaccatctcgacgagatcaaccagctgctcggcgtgcgcggcgccaacgcggaagatccggtcgcggtgatccgcacgcacgtgaaccggctcaagctgcagggcgtgtgatggcgcaggccgatcgtccggcgcgcggcgggctggccgcgcgcccgatgcgcggcgcgtcgttcgcgctggccgggctcgtcgcgtgtgccgcctgtgccgcggtcgtgctgtggcttcggcccgccgccccgtcgcccgcgccggccggtgccgtcgcgggcgggccggcggccggcgtgcccgccgcggcaagcggcgcggcggaggccgccatgccgttgccggcggcgctgccgggcgcgctggccggctcgcatgcgccgcgcctgccgctggccgccggcggcgggctcgcgaggacgcgcgcggtgcgcgagttcttcgactattgcctgaccgcgcagggcgaactgacgcccgccgcgctcgatgcgctggtgcggcgcgagatcgccgcgcagcttgacggcagccccgcgcaagcggaggcgctcggcgtctggcgccgctatcgcgcctacttcgacgcgctcgcgcaattgcccggcgacggcgcggtgctcggcgacaagctcgatccggccgccatgcagctcgcgctcgatcagcgcgcggcgctggccgaccgcacgctcggcgagtgggccgagccgttcttcggcgacgagcagcgccggcagcgccatgacctcgaacggatccggatcgccaacgacaccacgctgagccccgagcagaaggccgcgcggcttgccgcgctcgacgcgcagctgacgccggacgagcgcgcgcagcaggcggcgctgcatgcgcagcaggacgcggtgacgaagatcgccgacctgcagaaggccggcgcgacgcccgaccagatgcgcgcgcagatcgcgcagacgctcgggcccgaggcggccgcgcgcgccgcgcagatgcagcaggacgacgaggcgtggcagacgcgctatcaagcctatgcggccgagcgcgaccggatcgcggcgcaggggctcgcgccgcaggatcgcgatgcgcggatcgcgcagctcaggcagcagacttttacggcgccgggggaggcgatccgcgcggcgtcgctcgatcgcggcgcgggcggttag

SEQ ID NO: 68 - DNA, 35 bp, Artificial Sequence
  Primer
agcggaggtaaagcaatggtcagatcgatgcgttc

SEQ ID NO: 69 - DNA, 35 bp, Artificial Sequence
  Primer
gtcgaaaaccgcggcctaaccgcccgcgccgcgat

SEQ ID NO: 70 - DNA, 29 bp, Artificial Sequence
  Primer
tgctttacctccgctaagtggtgatgaac

SEQ ID NO: 71 - DNA, 25 bp, Artificial Sequence
  Primer
gccgcggttttcgactgcttcaaag

SEQ ID NO: 72 - DNA, 1095 bp, Burkholderia cepacia
atggccagatcgatgcgttccagggtggtggcaggggcagtggcatgcgcgatgagcgtcgcgccgttcgcggggacgaccgcggtgatgacgctcgcgacgacgcacgcggcgatggcggcgaccgcgcccgccgacaactacgcggcgacgcgttatccgatcatcctcgtgcacgggctcacgggcaccgacaagtacgcgggcgtgctcgagtactggtacggcatccaggaagacctgcagcagcgcggcgcgaccgtctacgtcgcgaacctgtcgggcttccagagcgacgacggcccgaacgggcgcggcgaacagttgctcgcgtacgtgaagacggtgcttgccgcgacgggcgcgaccaaggtcaatctcgtcggccacagccagggcgggctcacgtcgcgttacgtcgcggctgtcgcgccggatctcgtcgcgtcggtgacgacgatcggcacgccgcatcgcggctccgagttcgccgacttcgtgcagggcgtgctcgcatacgatccgaccgggctttcgtcaacggtgatcgcggcgttcgtcaatgtgttcggaatcctcacgagcagcagcaacaacacgaaccaggacgcgctcgcggcgctgaagacgctgacgaccgcccaggccgccacgtacaaccagaactatccgagcgcgggccttggcgcgccgggcagttgccagaccggcgcgccgacggaaaccgtcggcggcaacacgcatctgctgtattcgtgggccggcacggcgatccagccgacgatctccgtgttcggtgtcacgggcgcgacggacactagcacgattccgctcgtcgatccggcgaacgcgctcgacccgtcgacgcttgcgctgttcggcacgggcacggtgatggtcaaccgcggctcgggccagaacgacggggtcgtgtcgaaatgcagcgcgctgtacggccaggtgctgagcacgagctacaagtggaaccatctggacgagatcaaccagttgctcggcgtgcgcggcgcgaacgcggaagatccggtcgcggtgatccgcacgcatgcgaaccgtctgaagctggcgggcgtgtaa

SEQ ID NO: 73 - DNA, 35 bp, Artificial Sequence
  Primer
cgataaggacagcagatggccagatcgatgcgttc

SEQ ID NO: 74 - DNA, 35 bp, Artificial Sequence
  Primer
acgtgccgccatcgattacacgcccgccagcttca

SEQ ID NO: 75 - DNA, 35 bp, Artificial Sequence
  Primer
tcgatggcggcacgtgaagggcgcgcgccgctggc

SEQ ID NO: 76 - DNA, 35 bp, Artificial Sequence
  Primer
acgttggccagatctgtcgcgcgcggtgccgccgc

SEQ ID NO: 77 - DNA, 35 bp, Artificial Sequence
  Primer
catcgatctggccatctgctgtccttatcgtctga

SEQ ID NO: 78 - DNA, 35 bp, Artificial Sequence
  Primer
acgttggccagatctgctgccggcgaacctcgtgc

SEQ ID NO: 79 - DNA, 35 bp, Artificial Sequence
  Primer
catcgatctggccatgattacctccgggatttttt

SEQ ID NO: 80 - DNA, 20 bp, Artificial Sequence
  Primer
atggccagatcgatgcgttc

SEQ ID NO: 81 - DNA, 30 bp, Artificial Sequence
  Primer
agatctggccaacgtttgcgccctgactag

SEQ ID NO: 82 - DNA, 35 bp, Artificial Sequence
  Primer
acgttggccagatctcccgccagttgccggcgagc

SEQ ID NO: 83 - DNA, 35 bp, Artificial Sequence
  Primer
acgttggccagatctaggacggcgcacacgccggc

SEQ ID NO: 84 - DNA, 35 bp, Artificial Sequence
  Primer
acgttggccagatctgaaacggtcgattccgccag

SEQ ID NO: 85 - DNA, 35 bp, Artificial Sequence
  Primer
acgttggccagatctgccccgctttttcgaacttt

SEQ ID NO: 86 - DNA, 35 bp, Artificial Sequence
  Primer
acgttggccagatctttcgaactttactttttcga

SEQ ID NO: 87 - DNA, 35 bp, Artificial Sequence
  Primer
acgttggccagatctactttttcgatttcgttcgt

SEQ ID NO: 88 - DNA, 35 bp, Artificial Sequence
  Primer
acgttggccagatcttttcgttcgttaaatttcga

SEQ ID NO: 89 - DNA, 35 bp, Artificial Sequence
  Primer
acgttggccagatcttaaatttcgaattcgaacat

SEQ ID NO: 90 - DNA, 35 bp, Artificial Sequence
  Primer
acgttggccagatctattcgaacatttcgtgttca

SEQ ID NO: 91 - DNA, 35 bp, Artificial Sequence
  Primer
acgttggccagatctcgttcgagcgtaccgacaag

SEQ ID NO: 92 - DNA, 35 bp, Artificial Sequence
  Primer
acgttggccagatctccgcctcgcgggggcagcat

SEQ ID NO: 93 - DNA, 35 bp, Artificial Sequence
  Primer
acgttggccagatctttctctatcccggatgccgg

SEQ ID NO: 94 - DNA, 35 bp, Artificial Sequence
  Primer
acgttggccagatctcggatgccggcattgttggc

SEQ ID NO: 95 - DNA, 35 bp, Artificial Sequence
  Primer
acgttggccagatctcattgttggctccggggaaa

SEQ ID NO: 96 - DNA, 35 bp, Artificial Sequence
  Primer
acgttggccagatcttccggggaaacagtgttttc

SEQ ID NO: 97 - DNA, 35 bp, Artificial Sequence
  Primer
acgttggccagatctcagtgttttcgctctttcat

SEQ ID NO: 98 - DNA, 20 bp, Artificial Sequence
  Primer
atgacctcgattagcaaacg

SEQ ID NO: 99 - DNA, 28 bp, Artificial Sequence
  Primer
ttggccagtgtattcgctcctgttccag